European Patent Application EP 4 394 043 A1, published July 3, 2024. Title: METHOD FOR MODIFYING CELL. Applicant: CELLS & GENES BIOTECH (SHANGHAI) CO., LTD. The sequence listing filed with the application follows.

SEQUENCE LISTING (5 sequences)

SEQ ID NO: 1 - DNA, 3694 bp, synthetic construct
  misc_feature 1..3694: note = knock-in of GPC3 CAR-CD34 sequence at TRAC
  source 1..3694: mol_type = other DNA
cagtttgctttgctgggcctttttcccatgcctgcctttactctgccagagttatattgctggggttttgaagaagatcctattaaataaaagaataagcagtattattaagtagccctgcatttcaggtttccttgagtggcaggccaggcctggccgtgaacgttcactgaaatcatggcctcttggccaagattgatagcttgtgcctgtccctgagtcccagtccatcacgagcagctggtttctaagatgctatttcccgtataaagcatgagaccgtgacttgccagccccacagagccccgcccttgtccatcactggcatctggactccagcctgggttggggcaaagagggaaatgagatcatgtcctaaccctgatcctcttgtcccacactgacctcttctcttcctcccacagggcctcgagagatctggcagcggagagggcagaggaagtcttctaacatgcggtgacgtggaggagaatcccggccctaggctcgagatggccttaccagtgaccgccttgctcctgccgctggccttgctgctccacgccgccaggccgcaggtgcagctggtgcagtctggagctgaggtgaagaagcctggggcctcagtgaaggtctcctgcaaggcttctggatacaccttcaccgactatgaaatgcactgggtgcgacaggcccctggacaagggcttgagtggatgggagctcttgatcctaaaactggtgatactgcctacagtcagaagttcaagggcagagtcacgctgaccgcggacaaatccacgagcacagcctacatggagctgagcagcctgacatctgaggacacggccgtgtattactgtacaagattctactcctatacttactggggccagggaaccctggtcaccgtctcctcaggaggaggaggctctggaggaggagggagtggaggcgggggaagcgacgtggtgatgacccagagccccctgagcctgcccgtgacccccggcgagcccgccagcatcagctgcaggagcagccagagcctggtgcacagcaacggcaacacctacctgcactggtacctgcagaagcccggccagagcccccagctgctgatctacaaggtgagcaacaggttcagcggcgtgcccgacaggttcagcggcagcggcagcggcaccgacttcaccctgaagatcagcagggtggaggccgaggacgtgggcgtgtactactgcagccagaacacccacgtgccccccaccttcggccagggcaccaagctggagatcaagaccacgacgccagcgccgcgaccaccaacaccggcgcccaccatcgcgtcgcagcccctgtccctgcgcccagaggcgtgccggccagcggcggggggcgcagtgcacacgagggggctggacttcgcctgtgatatctacatctgggcgcccttggccgggacttgtggggtccttctcctgtcactggttatcaccctttactgcaaacggggcagaaagaaactcctgtatatattcaaacaaccatttatgagaccagtacaaactactcaagaggaagatggctgtagctgccgatttccagaagaagaagaaggaggatgtgaactgagagtgaagttcagcaggagcgcagacgcccccgcgtaccagcagggccagaaccagctctataacgagctcaatctaggacgaagagaggagtacgatgttttggacaagagacgtggccgggaccctgagatggggggaaagccgagaaggaagaaccctcaggaaggcctgtacaatgaactgcagaaagataagatggcggaggcctacagtgagattgggatgaaaggcgagcgccggaggggcaaggggcacgatggcctttaccagggtctcagtacagccaccaaggacacctacgacgcccttcacatgcaggccctgccccctcgcggcagcggcgccacaaacttctctctgctaaagcaagcaggtgatgttgaagaaaaccccgggcctatgctggtccgcaggggcgcgcgcgcagggcccaggatgccgcggggctggaccgcgctttgcttgctgagtttgctgccttctgggttcatgagtcttgacaacaacggtactgctaccccagagttacctacccagggaacattttcaaatgtttctacaaatgtatcctaccaagaaactacaacacctagtacccttggaagtaccagcctgcaccctgtgtctcaacatggcaatgaggccacaacaaacatcacagaaacgacagtcaaattcacatctacctctgtgataacctcagtttatggaaacacaaactcttctgtccagtcacagacctctgtaatcagcacagtgttcaccaccccagccaacgtttcaactccagagacaaccttgaagcctagcctgtcacctggaaatgtttcagacctttcaaccactagcactagccttgcaacatctcccactaaaccctatacatcatcttctcctatcctaagtgacatcaaggcagaaatcaaatgttcaggcatcagagaagtgaaattgactcagggcatctgcctggagcaaaataagacctccagctgtgcggagtttaagaaggacaggggagagggcctggcccgagtgctgtgtggggaggagcaggctgatgctgatgctggggcccaggtatgctccctgctccttgcccagtctgaggtgaggcctcagtgtctactgctggtcttggccaacagaacagaaatttccagcaaactccaacttatgaaaaagcaccaatctgacctgaaaaagctggggatcctagatttcactgagcaagatgttgcaagccaccagagctattcccaaaagaccctgattgcactggtcacctcgggagccctgctggctgtcttgggcatcactggctatttcctgatgaatcgccgcagctggagccccacaggagaaaggctggaactggagccttaactgtgccttctagttgccagccatctgttgtttgcccctcccccgtgccttccttgaccctggaaggtgccactcccactgtcctttcctaataaaatgaggaaattgcatcgcattgtctgagtaggtgtcattctattctggggggtggggtggggcaggacagcaagggggaggattgggaagacaatagcaggcatgctggggatgcggtgggctctatgggaattctctagaaatattctcgaggtttaaacgtcgacgcggccgcgatatccagaaccctgaccctgccgtgtaccagctgagagactctaaatccagtgacaagtctgtctgcctattcaccgattttgattctcaaacaaatgtgtcacaaagtaaggattctgatgtgtatatcacagacaaaactgtgctagacatgaggtctatggacttcaagagcaacagtgctgtggcctggagcaacaaatctgactttgcatgtgcaaacgccttcaacaacagcattattccagaagacaccttcttccccagcccaggtaagggcagctttggtgccttcgcaggctgtttccttgcttcaggaatggccaggttctgcccagagctctggtcaatgatgtctaaaactcctctgattggtggtctcggccttatccattgcc

SEQ ID NO: 2 - DNA, 3703 bp, synthetic construct
  misc_feature 1..3703: note = Knock-in of CD19 CAR-CD34 sequence at TRAC
  source 1..3703: mol_type = other DNA
cagtttgctttgctgggcctttttcccatgcctgcctttactctgccagagttatattgctggggttttgaagaagatcctattaaataaaagaataagcagtattattaagtagccctgcatttcaggtttccttgagtggcaggccaggcctggccgtgaacgttcactgaaatcatggcctcttggccaagattgatagcttgtgcctgtccctgagtcccagtccatcacgagcagctggtttctaagatgctatttcccgtataaagcatgagaccgtgacttgccagccccacagagccccgcccttgtccatcactggcatctggactccagcctgggttggggcaaagagggaaatgagatcatgtcctaaccctgatcctcttgtcccacactgacctcttctcttcctcccacagggcctcgagagatctggcagcggagagggcagaggaagtcttctaacatgcggtgacgtggaggagaatcccggccctaggctcgagatggccttaccagtgaccgccttgctcctgccgctggccttgctgctccacgccgccaggccggacatccagatgacacagactacatcctccctgtctgcctctctgggagacagagtcaccatcagttgcagggcaagtcaggacattagtaaatatttaaattggtatcagcagaaaccagatggaactgttaaactcctgatctaccatacatcaagattacactcaggagtcccatcaaggttcagtggcagtgggtctggaacagattattctctcaccattagcaacctggagcaagaagatattgccacttacttttgccaacagggtaatacgcttccgtacacgttcggaggggggactaagttggaaataacaggctccacctctggatccggcaagcccggatctggcgagggatccaccaagggcgaggtgaaactgcaggagtcaggacctggcctggtggcgccctcacagagcctgtccgtcacatgcactgtctcaggggtctcattacccgactatggtgtaagctggattcgccagcctccacgaaagggtctggagtggctgggagtaatatggggtagtgaaaccacatactataattcagctctcaaatccagactgaccatcatcaaggacaactccaagagccaagttttcttaaaaatgaacagtctgcaaactgatgacacagccatttactactgtgccaaacattattactacggtggtagctatgctatggactactggggtcaaggaacctcagtcaccgtctcctcaaccacaacccctgcccctagacctcctacacccgcccctacaatcgccagccagcctctgtctctgaggcccgaggcttgtagacctgctgctggcggagccgtgcacaccagaggactggatttcgcctgcgacatctacatctgggcccctctggccggcacatgtggcgtgctgctgctgagcctcgtgatcaccctgtactgcaagcggggcagaaagaagctgctgtacatcttcaagcagcccttcatgcggcccgtgcagaccacccaggaagaggacggctgctcctgcagattccccgaggaagaagaaggcggctgcgagctgagagtgaagttcagcagaagcgccgacgcccctgcctatcagcagggccagaaccagctgtacaacgagctgaacctgggcagacgggaagagtacgatgtgctggacaaaagacgtggccgggaccctgagatggggggaaagccgagaaggaagaaccctcaggaaggcctgtacaatgaactgcagaaagataagatggcggaggcctacagtgagattgggatgaaaggcgagcgccggaggggcaaggggcacgatggcctttaccagggtctcagtacagccaccaaggacacctacgacgcccttcacatgcaggccctgccccctcgcggcagcggcgccacaaacttctctctgctaaagcaagcaggtgatgttgaagaaaaccccgggcctatgctggtccgcaggggcgcgcgcgcagggcccaggatgccgcggggctggaccgcgctttgcttgctgagtttgctgccttctgggttcatgagtcttgacaacaacggtactgctaccccagagttacctacccagggaacattttcaaatgtttctacaaatgtatcctaccaagaaactacaacacctagtacccttggaagtaccagcctgcaccctgtgtctcaacatggcaatgaggccacaacaaacatcacagaaacgacagtcaaattcacatctacctctgtgataacctcagtttatggaaacacaaactcttctgtccagtcacagacctctgtaatcagcacagtgttcaccaccccagccaacgtttcaactccagagacaaccttgaagcctagcctgtcacctggaaatgtttcagacctttcaaccactagcactagccttgcaacatctcccactaaaccctatacatcatcttctcctatcctaagtgacatcaaggcagaaatcaaatgttcaggcatcagagaagtgaaattgactcagggcatctgcctggagcaaaataagacctccagctgtgcggagtttaagaaggacaggggagagggcctggcccgagtgctgtgtggggaggagcaggctgatgctgatgctggggcccaggtatgctccctgctccttgcccagtctgaggtgaggcctcagtgtctactgctggtcttggccaacagaacagaaatttccagcaaactccaacttatgaaaaagcaccaatctgacctgaaaaagctggggatcctagatttcactgagcaagatgttgcaagccaccagagctattcccaaaagaccctgattgcactggtcacctcgggagccctgctggctgtcttgggcatcactggctatttcctgatgaatcgccgcagctggagccccacaggagaaaggctggaactggagccttaactgtgccttctagttgccagccatctgttgtttgcccctcccccgtgccttccttgaccctggaaggtgccactcccactgtcctttcctaataaaatgaggaaattgcatcgcattgtctgagtaggtgtcattctattctggggggtggggtggggcaggacagcaagggggaggattgggaagacaatagcaggcatgctggggatgcggtgggctctatgggaattctctagaaatattctcgaggtttaaacgtcgacgcggccgcgatatccagaaccctgaccctgccgtgtaccagctgagagactctaaatccagtgacaagtctgtctgcctattcaccgattttgattctcaaacaaatgtgtcacaaagtaaggattctgatgtgtatatcacagacaaaactgtgctagacatgaggtctatggacttcaagagcaacagtgctgtggcctggagcaacaaatctgactttgcatgtgcaaacgccttcaacaacagcattattccagaagacaccttcttccccagcccaggtaagggcagctttggtgccttcgcaggctgtttccttgcttcaggaatggccaggttctgcccagagctctggtcaatgatgtctaaaactcctctgattggtggtctcggccttatccattgcc

SEQ ID NO: 3 - DNA, 1527 bp, synthetic construct
  misc_feature 1..1527: note = nucleic acid molecule encoding GPC3 CAR
  source 1..1527: mol_type = other DNA
atggccttaccagtgaccgccttgctcctgccgctggccttgctgctccacgccgccaggccgcaggtgcagctggtgcagtctggagctgaggtgaagaagcctggggcctcagtgaaggtctcctgcaaggcttctggatacaccttcaccgactatgaaatgcactgggtgcgacaggcccctggacaagggcttgagtggatgggagctcttgatcctaaaactggtgatactgcctacagtcagaagttcaagggcagagtcacgctgaccgcggacaaatccacgagcacagcctacatggagctgagcagcctgacatctgaggacacggccgtgtattactgtacaagattctactcctatacttactggggccagggaaccctggtcaccgtctcctcaggaggaggaggctctggaggaggagggagtggaggcgggggaagcgacgtggtgatgacccagagccccctgagcctgcccgtgacccccggcgagcccgccagcatcagctgcaggagcagccagagcctggtgcacagcaacggcaacacctacctgcactggtacctgcagaagcccggccagagcccccagctgctgatctacaaggtgagcaacaggttcagcggcgtgcccgacaggttcagcggcagcggcagcggcaccgacttcaccctgaagatcagcagggtggaggccgaggacgtgggcgtgtactactgcagccagaacacccacgtgccccccaccttcggccagggcaccaagctggagatcaagaccacgacgccagcgccgcgaccaccaacaccggcgcccaccatcgcgtcgcagcccctgtccctgcgcccagaggcgtgccggccagcggcggggggcgcagtgcacacgagggggctggacttcgcctgtgatatctacatctgggcgcccttggccgggacttgtggggtccttctcctgtcactggttatcaccctttactgcaaacggggcagaaagaaactcctgtatatattcaaacaaccatttatgagaccagtacaaactactcaagaggaagatggctgtagctgccgatttccagaagaagaagaaggaggatgtgaactgagagtgaagttcagcaggagcgcagacgcccccgcgtaccagcagggccagaaccagctctataacgagctcaatctaggacgaagagaggagtacgatgttttggacaagagacgtggccgggaccctgagatggggggaaagccgagaaggaagaaccctcaggaaggcctgtacaatgaactgcagaaagataagatggcggaggcctacagtgagattgggatgaaaggcgagcgccggaggggcaaggggcacgatggcctttaccagggtctcagtacagccaccaaggacacctacgacgcccttcacatgcaggccctgccccctcgcggcagcggcgccacaaacttctctctgctaaagcaagcaggtgatgttgaagaaaaccccgggccttaa

SEQ ID NO: 4 - DNA, 987 bp, synthetic construct
  misc_feature 1..987: note = nucleic acid molecule encoding CD34
  source 1..987: mol_type = other DNA
atgctggtccgcaggggcgcgcgcgcagggcccaggatgccgcggggctggaccgcgctttgcttgctgagtttgctgccttctgggttcatgagtcttgacaacaacggtactgctaccccagagttacctacccagggaacattttcaaatgtttctacaaatgtatcctaccaagaaactacaacacctagtacccttggaagtaccagcctgcaccctgtgtctcaacatggcaatgaggccacaacaaacatcacagaaacgacagtcaaattcacatctacctctgtgataacctcagtttatggaaacacaaactcttctgtccagtcacagacctctgtaatcagcacagtgttcaccaccccagccaacgtttcaactccagagacaaccttgaagcctagcctgtcacctggaaatgtttcagacctttcaaccactagcactagccttgcaacatctcccactaaaccctatacatcatcttctcctatcctaagtgacatcaaggcagaaatcaaatgttcaggcatcagagaagtgaaattgactcagggcatctgcctggagcaaaataagacctccagctgtgcggagtttaagaaggacaggggagagggcctggcccgagtgctgtgtggggaggagcaggctgatgctgatgctggggcccaggtatgctccctgctccttgcccagtctgaggtgaggcctcagtgtctactgctggtcttggccaacagaacagaaatttccagcaaactccaacttatgaaaaagcaccaatctgacctgaaaaagctggggatcctagatttcactgagcaagatgttgcaagccaccagagctattcccaaaagaccctgattgcactggtcacctcgggagccctgctggctgtcttgggcatcactggctatttcctgatgaatcgccgcagctggagccccacaggagaaaggctggaactggagccttaa

SEQ ID NO: 5 - DNA, 1410 bp, synthetic construct
  misc_feature 1..1410: note = nucleic acid molecule encoding CD19 CAR
  source 1..1410: mol_type = other DNA
atggacatccagatgacacagactacatcctccctgtctgcctctctgggagacagagtcaccatcagttgcagggcaagtcaggacattagtaaatatttaaattggtatcagcagaaaccagatggaactgttaaactcctgatctaccatacatcaagattacactcaggagtcccatcaaggttcagtggcagtgggtctggaacagattattctctcaccattagcaacctggagcaagaagatattgccacttacttttgccaacagggtaatacgcttccgtacacgttcggaggggggactaagttggaaataacaggctccacctctggatccggcaagcccggatctggcgagggatccaccaagggcgaggtgaaactgcaggagtcaggacctggcctggtggcgccctcacagagcctgtccgtcacatgcactgtctcaggggtctcattacccgactatggtgtaagctggattcgccagcctccacgaaagggtctggagtggctgggagtaatatggggtagtgaaaccacatactataattcagctctcaaatccagactgaccatcatcaaggacaactccaagagccaagttttcttaaaaatgaacagtctgcaaactgatgacacagccatttactactgtgccaaacattattactacggtggtagctatgctatggactactggggtcaaggaacctcagtcaccgtctcctcaaccacaacccctgcccctagacctcctacacccgcccctacaatcgccagccagcctctgtctctgaggcccgaggcttgtagacctgctgctggcggagccgtgcacaccagaggactggatttcgcctgcgacatctacatctgggcccctctggccggcacatgtggcgtgctgctgctgagcctcgtgatcaccctgtactgcaagcggggcagaaagaagctgctgtacatcttcaagcagcccttcatgcggcccgtgcagaccacccaggaagaggacggctgctcctgcagattccccgaggaagaagaaggcggctgcgagctgagagtgaagttcagcagaagcgccgacgcccctgcctatcagcagggccagaaccagctgtacaacgagctgaacctgggcagacgggaagagtacgatgtgctggacaaaagacgtggccgggaccctgagatggggggaaagccgagaaggaagaaccctcaggaaggcctgtacaatgaactgcagaaagataagatggcggaggcctacagtgagattgggatgaaaggcgagcgccggaggggcaaggggcacgatggcctttaccagggtctcagtacagccaccaaggacacctacgacgcccttcacatgcaggccctgccccctcgctaa